European Patent Specification EP 3 402 817 B1, published October 18, 2023. Title: ANTI-N3pGlu AMYLOID BETA PEPTIDE ANTIBODIES AND USES THEREOF. Applicant: Eli Lilly and Company. The sequence listing filed with the application follows.

SEQUENCE LISTING (17 sequences)

SEQ ID NO: 1 - protein, 13 aa, Artificial Sequence
  Synthetic Construct
KASGYTFTDYYIN

SEQ ID NO: 2 - protein, 17 aa, Artificial Sequence
  Synthetic Construct
WINPGSGNTKYNEKFKG

SEQ ID NO: 3 - protein, 8 aa, Artificial Sequence
  Synthetic Construct
TREGETVY

SEQ ID NO: 4 - protein, 16 aa, Artificial Sequence
  Synthetic Construct
KSSQSLLYSRGKTYLN

SEQ ID NO: 5 - protein, 8 aa, Artificial Sequence
  Synthetic Construct
YAVSKLDS

SEQ ID NO: 6 - protein, 8 aa, Artificial Sequence
  Synthetic Construct
YDVSKLDS

SEQ ID NO: 7 - protein, 9 aa, Artificial Sequence
  Synthetic Construct
VQGTHYPFT

SEQ ID NO: 8 - protein, 115 aa, Artificial Sequence
  Synthetic Construct
QVQLVQSGAEVKKPGSSVKVSCKASGYTFTDYYINWVRQAPGQGLEWMGWINPGSGNTKYNEKFKGRVTITADESTSTAYMELSSLRSEDTAVYYCTREGETVYWGQGTLVTVSS

SEQ ID NO: 9 - protein, 112 aa, Artificial Sequence
  Synthetic Construct
DVVMTQSPLSLPVTLGQPASISCKSSQSLLYSRGKTYLNWFQQRPGQSPRRLIYDVSKLDSGVPDRFSGSGSGTDFTLKISRVEAEDVGVYYCVQGTHYPFTFGQGTKLEIK

SEQ ID NO: 10 - protein, 112 aa, Artificial Sequence
  Synthetic Construct
DIQMTQSPSTLSASVGDRVTITCKSSQSLLYSRGKTYLNWLQQKPGKAPKLLIYAVSKLDSGVPSRFSGSGSGTEFTLTISSLQPDDFATYYCVQGTHYPFTFGQGTKLEIK

SEQ ID NO: 11 - protein, 444 aa, Artificial Sequence
  Synthetic Construct
QVQLVQSGAEVKKPGSSVKVSCKASGYTFTDYYINWVRQAPGQGLEWMGWINPGSGNTKYNEKFKGRVTITADESTSTAYMELSSLRSEDTAVYYCTREGETVYWGQGTLVTVSSASTKGPSVFPLAPSSKSTSGGTAALGCLVKDYFPEPVTVSWNSGALTSGVHTFPAVLQSSGLYSLSSVVTVPSSSLGTQTYICNVNHKPSNTKVDKKVEPKSCDKTHTCPPCPAPELLGGPSVFLFPPKPKDTLMISRTPEVTCVVVDVSHEDPEVKFNWYVDGVEVHNAKTKPREEQYNSTYRVVSVLTVLHQDWLNGKEYKCKVSNKALPAPIEKTISKAKGQPREPQVYTLPPSRDELTKNQVSLTCLVKGFYPSDIAVEWESNGQPENNYKTTPPVLDSDGSFFLYSKLTVDKSRWQQGNVFSCSVMHEALHNHYTQKSLSLSPG

SEQ ID NO: 12 - protein, 219 aa, Artificial Sequence
  Artifical Sequence
DVVMTQSPLSLPVTLGQPASISCKSSQSLLYSRGKTYLNWFQQRPGQSPRRLIYDVSKLDSGVPDRFSGSGSGTDFTLKISRVEAEDVGVYYCVQGTHYPFTFGQGTKLEIKRTVAAPSVFIFPPSDEQLKSGTASVVCLLNNFYPREAKVQWKVDNALQSGNSQESVTEQDSKDSTYSLSSTLTLSKADYEKHKVYACEVTHQGLSSPVTKSFNRGEC

SEQ ID NO: 13 - protein, 219 aa, Artificial Sequence
  Artifical Sequence
DIQMTQSPSTLSASVGDRVTITCKSSQSLLYSRGKTYLNWLQQKPGKAPKLLIYAVSKLDSGVPSRFSGSGSGTEFTLTISSLQPDDFATYYCVQGTHYPFTFGQGTKLEIKRTVAAPSVFIFPPSDEQLKSGTASVVCLLNNFYPREAKVQWKVDNALQSGNSQESVTEQDSKDSTYSLSSTLTLSKADYEKHKVYACEVTHQGLSSPVTKSFNRGEC

SEQ ID NO: 14 - DNA, 1332 bp, Artificial Sequence
  Synthetic Construct
caggtgcagctggtgcagtctggggctgaggtgaagaagcctgggtcctcggtgaaggtctcctgcaaggcttctggatacaccttcaccgactattatatcaactgggtgcgacaggcccctggacaagggcttgagtggatgggatggatcaaccctggcagtggtaatacaaagtacaatgagaagttcaagggcagagtcacgattaccgcggacgaatccacgagcacagcctacatggagctgagcagcctgagatctgaggacacggccgtgtattactgtacaagagaaggcgagacggtctactggggccagggaaccctggtcaccgtctcctcagcctccaccaagggcccatcggtcttcccgctagcaccctcctccaagagcacctctgggggcacagcggccctgggctgcctggtcaaggactacttccccgaaccggtgacggtgtcgtggaactcaggcgccctgaccagcggcgtgcacaccttcccggctgtcctacagtcctcaggactctactccctcagcagcgtggtgaccgtgccctccagcagcttgggcacccagacctacatctgcaacgtgaatcacaagcccagcaacaccaaggtggacaagaaagttgagcccaaatcttgtgacaaaactcacacatgcccaccgtgcccagcacctgaactcctggggggaccgtcagtcttcctcttccccccaaaacccaaggacaccctcatgatctcccggacccctgaggtcacatgcgtggtggtggacgtgagccacgaagaccctgaggtcaagttcaactggtacgtggacggcgtggaggtgcataatgccaagacaaagccgcgggaggagcagtacaacagcacgtaccgtgtggtcagcgtcctcaccgtcctgcaccaggactggctgaatggcaaggagtacaagtgcaaggtctccaacaaagccctcccagcccccatcgagaaaaccatctccaaagccaaagggcagccccgagaaccacaggtgtacaccctgcccccatcccgggacgagctgaccaagaaccaggtcagcctgacctgcctggtcaaaggcttctatcccagcgacatcgccgtggagtgggagagcaatgggcagccggagaacaactacaagaccacgccccccgtgctggactccgacggctccttcttcctctatagcaagctcaccgtggacaagagcaggtggcagcaggggaacgtcttctcatgctccgtgatgcatgaggctctgcacaaccactacacgcagaagagcctctccctgtctccgggt

SEQ ID NO: 15 - DNA, 657 bp, Artificial Sequence
  Synthetic Construct
gatgttgtgatgactcagtctccactctccctgcccgtcacccttggacagccggcctccatctcctgcaagtctagtcaaagcctcctgtacagtcgcggaaaaacctacttgaattggtttcagcagaggccaggccaatctccaaggcgcctaatttatgatgtttctaaactggactctggggtcccagacagattcagcggcagtgggtcaggcactgatttcacactgaaaatcagcagggtggaggctgaggatgttggggtttattactgcgtgcaaggtacacactaccctttcacttttggccaagggaccaagctggagatcaaacggaccgtggctgcaccatctgtcttcatcttcccgccatctgatgagcagttgaaatctggaactgcctctgttgtgtgcctgctgaataacttctatcccagagaggccaaagtacagtggaaggtggataacgccctccaatcgggtaactcccaggagagtgtcacagagcaggacagcaaggacagcacctacagcctcagcagcaccctgacgctgagcaaagcagactacgagaaacacaaagtctacgcctgcgaagtcacccatcagggcctgagctcgcccgtcacaaagagcttcaacaggggagagtgc

SEQ ID NO: 16 - DNA, 657 bp, Artificial Sequence
  Synthetic Construct
gacatccagatgacccagtctccttccaccctgtctgcatctgtaggagacagagtcaccatcacttgcaagtccagtcagagtctcctgtacagtcgcggaaaaacctatttgaactggctccagcagaaaccagggaaagcccctaagctcctgatctatgctgtctccaaactggacagtggggtcccatcaaggttcagcggcagtggatctgggacagaattcactctcaccatcagcagcctgcagcctgatgattttgcaacttattactgcgtgcagggtacacattatcctttcacttttggccaggggaccaagctggagatcaaacggaccgtggctgcaccatctgtcttcatcttcccgccatctgatgagcagttgaaatctggaactgcctctgttgtgtgcctgctgaataacttctatcccagagaggccaaagtacagtggaaggtggataacgccctccaatcgggtaactcccaggagagtgtcacagagcaggacagcaaggacagcacctacagcctcagcagcaccctgacgctgagcaaagcagactacgagaaacacaaagtctacgcctgcgaagtcacccatcagggcctgagctcgcccgtcacaaagagcttcaacaggggagagtgc

SEQ ID NO: 17 - protein, 40 aa, Artificial Sequence
  Synthetic Construct
  MISC_FEATURE (1)..(1): Xaa at position 1 = pyroglutamic acid
XFRHDSGYEVHHQKLVFFAEDVGSNKGAIIGLMVGGVVIA